European Patent Application EP 4 427 755 A1, published September 11, 2024. Title: 살모넬라 균주 및 면역관문억제제를 유효성분으로 포함하는 암의 예방 또는 치료용 약학조성물. Applicant: 전남대학교 산학협력단. Application KR. The sequence listing filed with the application follows.

SEQUENCE LISTING (4 sequences)

SEQ ID NO: 1 - protein, 305 aa, synthetic construct
MIMTGIFAEQTVEVVKSAIETADGALDLYNKYLDQVIPWKTFDETIKELSRFKQEYSQEASVLVGDIKVLLMDSQDKYFEATQTVYEWCGVVTQLLSAYILLFDEYNEKKASAQKDILIRILDDGVKKLNEAQKSLLTSSQSFNNASGKLLALDSQLTNDFSEKSSYFQSQVDRIRKEAYAGAAAGIVAGPFGLIISYSIAAGVIEGKLIPELNNRLKTVQNFFTSLSATVKQANKDIDAAKLKLATEIAAIGEIKTETETTRFYVDYDDLMLSLLKGAAKKMINTCNEYQQRHGKKTLFEVPDV

SEQ ID NO: 2-3 - skipped (2 entries)

SEQ ID NO: 4 - DNA, 192 bp, synthetic construct
  source 1..192: mol_type = other DNA
aagctgttgtgaccgcttgctctagccagctatcgagttgtgaaccgatccatctagcaattggtctcgatctagcgataggcttcgatctagctatgtagaaacgccgtgtgctcgatcgcctgacgctttttatcgcaactctctactgttgcttcaacagaacatattgactatccggtattacccggc